European Patent Specification EP 3 683 313 B1, published February 11, 2026. Title: Mutated Glycine Oxidase derived from Bucillus family. Applicant: NIPRO CORPORATION. The sequence listing filed with the application follows.

SEQUENCE LISTING (4 sequences)

SEQ ID NO: 1 - protein, 377 aa, Geobacillus kaustophilius HTA426
MTHRYDVAIVGGGVIGAAIGFELAKRRHRVAIFEKGTMGSGASSAAAGMLGAQSEFSTSSPLVPLALQSRALMPALAEELRERTGIDIGLVEKGLIKLATTEEEADDLYRHYTFWRGIGEPVQWLTKGEALEMEPRLAAEALAGAMYIPGDGQVSAPDLAAALAYAAASAGACLYEYTEVFDIRSDSSGHVLDTTGGTFAAEAVVIASGAWAARLGARVGLSLSVYPVKGECVMVRAPVPLLQTTVFAKNGCYIVPKSGNRLLIGATSTPGTFDRRVSAGGVMNLLHRAAHLVPDIEQAEWVASWSGIRPQTEDGLPYLGEHPERRGLFVAAGHYRNGILLSPLTGLLVADLVERKETAFDLAPFSLTRHIGKVGVE

SEQ ID NO: 2 - DNA, 1134 bp, Geobacillus kaustophilus HTA426
atgacgcatcggtatgacgtcgccatcgtcggcggcggggtgattggggcggccatcggttttgagctcgccaagcggcggcatcgcgtcgccatttttgaaaaaggaacgatgggaagcggggcgtcaagcgcggcagccggcatgcttggggcgcaatccgagttttcgacgtcaagcccgcttgtgccgcttgccttgcaaagccgagctctcatgccggccttggctgaagagctgagggagaggaccggcatcgatatcggccttgtcgaaaaaggattgatcaaactagcgacaacggaagaggaagcagacgatctctatcgccattatacattttggcggggcataggcgaaccggtgcagtggctcacgaaaggggaggcgcttgaaatggagccgcgtcttgcggcggaagcgcttgccggcgcgatgtacatccctggcgatgggcaagtgagcgctccggatttggccgccgctcttgcctatgccgccgcctccgccggcgcttgtctgtacgagtatacggaagtgttcgacatccgttccgacagcagtgggcatgtgttagacacaacaggcgggacgtttgccgccgaggcggtcgtcatcgcttccggcgcttgggcggcgcggctcggcgcgcgggtcgggctttcgctttccgtttatccggtcaaaggagaatgcgtcatggtgcgcgccccggttccgttgttgcaaacgactgtatttgcgaaaaacggctgctacatcgttccgaaatcaggaaaccggctgctcatcggagcgacgtccacgcccggcacgttcgatcgacgtgtatcggccggtggggtgatgaacttgcttcaccgcgccgcccaccttgttccggacatcgaacaggcggaatgggtggcatcatggagcggcattcggccgcagaccgaagacggcttgccttatctaggcgagcatccggagcggcgcggcttattcgtcgctgccggccattaccggaacggcattttgctcagcccattgaccggtctgcttgtcgccgacttagtggagcggaaagagacggcgtttgatcttgcgccattttcgttgacacgccatatcggaaaggtgggggtggaatga

SEQ ID NO: 3 - protein, 377 aa, Artificial Sequence
  The 251st amino acid in SEQ ID No.1 is an arbitrary amino acid.
MTHRYDVAIVGGGVIGAAIGFELAKRRHRVAIFEKGTMGSGASSAAAGMLGAQSEFSTSSPLVPLALQSRALMPALAEELRERTGIDIGLVEKGLIKLATTEEEADDLYRHYTFWRGIGEPVQWLTKGEALEMEPRLAAEALAGAMYIPGDGQVSAPDLAAALAYAAASAGACLYEYTEVFDIRSDSSGHVLDTTGGTFAAEAVVIASGAWAARLGARVGLSLSVYPVKGECVMVRAPVPLLQTTVFAKNXCYIVPKSGNRLLIGATSTPGTFDRRVSAGGVMNLLHRAAHLVPDIEQAEWVASWSGIRPQTEDGLPYLGEHPERRGLFVAAGHYRNGILLSPLTGLLVADLVERKETAFDLAPFSLTRHIGKVGVE

SEQ ID NO: 4 - DNA, 1134 bp, Artificial Sequence
  The 751st-753rd nucreotides in SEQ ID No.2 are arbitrary nucreotides.
atgacgcatcggtatgacgtcgccatcgtcggcggcggggtgattggggcggccatcggttttgagctcgccaagcggcggcatcgcgtcgccatttttgaaaaaggaacgatgggaagcggggcgtcaagcgcggcagccggcatgcttggggcgcaatccgagttttcgacgtcaagcccgcttgtgccgcttgccttgcaaagccgagctctcatgccggccttggctgaagagctgagggagaggaccggcatcgatatcggccttgtcgaaaaaggattgatcaaactagcgacaacggaagaggaagcagacgatctctatcgccattatacattttggcggggcataggcgaaccggtgcagtggctcacgaaaggggaggcgcttgaaatggagccgcgtcttgcggcggaagcgcttgccggcgcgatgtacatccctggcgatgggcaagtgagcgctccggatttggccgccgctcttgcctatgccgccgcctccgccggcgcttgtctgtacgagtatacggaagtgttcgacatccgttccgacagcagtgggcatgtgttagacacaacaggcgggacgtttgccgccgaggcggtcgtcatcgcttccggcgcttgggcggcgcggctcggcgcgcgggtcgggctttcgctttccgtttatccggtcaaaggagaatgcgtcatggtgcgcgccccggttccgttgttgcaaacgactgtatttgcgaaaaacnnntgctacatcgttccgaaatcaggaaaccggctgctcatcggagcgacgtccacgcccggcacgttcgatcgacgtgtatcggccggtggggtgatgaacttgcttcaccgcgccgcccaccttgttccggacatcgaacaggcggaatgggtggcatcatggagcggcattcggccgcagaccgaagacggcttgccttatctaggcgagcatccggagcggcgcggcttattcgtcgctgccggccattaccggaacggcattttgctcagcccattgaccggtctgcttgtcgccgacttagtggagcggaaagagacggcgtttgatcttgcgccattttcgttgacacgccatatcggaaaggtgggggtggaatga